European Patent Application EP 4 316 513 A1, published February 7, 2024. Title: NEW DNA SARS-CoV-2 VACCINE. Applicant: Consejo Superior de Investigaciones Cientificas. The sequence listing filed with the application follows.

SEQUENCE LISTING (32 sequences)

SEQ ID NO: 1 - protein, 1273 aa, synthetic construct
MFVFLVLLPLVSSQCVNLTTRTQLPPAYTNSFTRGVYYPDKVFRSSVLHSTQDLFLPFFSNVTWFHAIHVSGTNGTKRFDNPVLPFNDGVYFASTEKSNIIRGWIFGTTLDSKTQSLLIVNNATNVVIKVCEFQFCNDPFLGVYYHKNNKSWMESEFRVYSSANNCTFEYVSQPFLMDLEGKQGNFKNLREFVFKNIDGYFKIYSKHTPINLVRDLPQGFSALEPLVDLPIGINITRFQTLLALHRSYLTPGDSSSGWTAGAAAYYVGYLQPRTFLLKYNENGTITDAVDCALDPLSETKCTLKSFTVEKGIYQTSNFRVQPTESIVRFPNITNLCPFGEVFNATRFASVYAWNRKRISNCVADYSVLYNSASFSTFKCYGVSPTKLNDLCFTNVYADSFVIRGDEVRQIAPGQTGKIADYNYKLPDDFTGCVIAWNSNNLDSKVGGNYNYLYRLFRKSNLKPFERDISTEIYQAGSTPCNGVEGFNCYFPLQSYGFQPTNGVGYQPYRVVVLSFELLHAPATVCGPKKSTNLVKNKCVNFNFNGLTGTGVLTESNKKFLPFQQFGRDIADTTDAVRDPQTLEILDITPCSFGGVSVITPGTNTSNQVAVLYQDVNCTEVPVAIHADQLTPTWRVYSTGSNVFQTRAGCLIGAEHVNNSYECDIPIGAGICASYQTQTNSPRRARSVASQSIIAYTMSLGAENSVAYSNNSIAIPTNFTISVTTEILPVSMTKTSVDCTMYICGDSTECSNLLLQYGSFCTQLNRALTGIAVEQDKNTQEVFAQVKQIYKTPPIKDFGGFNFSQILPDPSKPSKRSFIEDLLFNKVTLADAGFIKQYGDCLGDIAARDLICAQKFNGLTVLPPLLTDEMIAQYTSALLAGTITSGWTFGAGAALQIPFAMQMAYRFNGIGVTQNVLYENQKLIANQFNSAIGKIQDSLSSTASALGKLQDVVNQNAQALNTLVKQLSSNFGAISSVLNDILSRLDKVEAEVQIDRLITGRLQSLQTYVTQQLIRAAEIRASANLAATKMSECVLGQSKRVDFCGKGYHLMSFPQSAPHGVVFLHVTYVPAQEKNFTTAPAICHDGKAHFPREGVFVSNGTHWFVTQRNFYEPQIITTDNTFVSGNCDVVIGIVNNTVYDPLQPELDSFKEELDKYFKNHTSPDVDLGDISGINASVVNIQKEIDRLNEVAKNLNESLIDLQELGKYEQYIKWPWYIWLGFIAGLIAIVMVTIMLCCMTSCCSCLKGCCSCGSCCKFDEDDSEPVLKGVKLHYT

SEQ ID NO: 2 - protein, 1273 aa, synthetic construct
  REGION 1..1273: note = Furin-stabilized S protein (Sfs)
MFVFLVLLPLVSSQCVNLTTRTQLPPAYTNSFTRGVYYPDKVFRSSVLHSTQDLFLPFFSNVTWFHAIHVSGTNGTKRFDNPVLPFNDGVYFASTEKSNIIRGWIFGTTLDSKTQSLLIVNNATNVVIKVCEFQFCNDPFLGVYYHKNNKSWMESEFRVYSSANNCTFEYVSQPFLMDLEGKQGNFKNLREFVFKNIDGYFKIYSKHTPINLVRDLPQGFSALEPLVDLPIGINITRFQTLLALHRSYLTPGDSSSGWTAGAAAYYVGYLQPRTFLLKYNENGTITDAVDCALDPLSETKCTLKSFTVEKGIYQTSNFRVQPTESIVRFPNITNLCPFGEVFNATRFASVYAWNRKRISNCVADYSVLYNSASFSTFKCYGVSPTKLNDLCFTNVYADSFVIRGDEVRQIAPGQTGKIADYNYKLPDDFTGCVIAWNSNNLDSKVGGNYNYLYRLFRKSNLKPFERDISTEIYQAGSTPCNGVEGFNCYFPLQSYGFQPTNGVGYQPYRVVVLSFELLHAPATVCGPKKSTNLVKNKCVNFNFNGLTGTGVLTESNKKFLPFQQFGRDIADTTDAVRDPQTLEILDITPCSFGGVSVITPGTNTSNQVAVLYQDVNCTEVPVAIHADQLTPTWRVYSTGSNVFQTRAGCLIGAEHVNNSYECDIPIGAGICASYQTQTNSPGGSGSVASQSIIAYTMSLGAENSVAYSNNSIAIPTNFTISVTTEILPVSMTKTSVDCTMYICGDSTECSNLLLQYGSFCTQLNRALTGIAVEQDKNTQEVFAQVKQIYKTPPIKDFGGFNFSQILPDPSKPSKRSFIEDLLFNKVTLADAGFIKQYGDCLGDIAARDLICAQKFNGLTVLPPLLTDEMIAQYTSALLAGTITSGWTFGAGAALQIPFAMQMAYRFNGIGVTQNVLYENQKLIANQFNSAIGKIQDSLSSTASALGKLQDVVNQNAQALNTLVKQLSSNFGAISSVLNDILSRLDKVEAEVQIDRLITGRLQSLQTYVTQQLIRAAEIRASANLAATKMSECVLGQSKRVDFCGKGYHLMSFPQSAPHGVVFLHVTYVPAQEKNFTTAPAICHDGKAHFPREGVFVSNGTHWFVTQRNFYEPQIITTDNTFVSGNCDVVIGIVNNTVYDPLQPELDSFKEELDKYFKNHTSPDVDLGDISGINASVVNIQKEIDRLNEVAKNLNESLIDLQELGKYEQYIKWPWYIWLGFIAGLIAIVMVTIMLCCMTSCCSCLKGCCSCGSCCKFDEDDSEPVLKGVKLHYT

SEQ ID NO: 3 - protein, 419 aa, synthetic construct
  REGION 1..419: note = Protein N amino acid sequence (Wuhan-Hu-1 strain). NCBI NC045512.2. Protein ID YP_009724397.2
MSDNGPQNQRNAPRITFGGPSDSTGSNQNGERSGARSKQRRPQGLPNNTASWFTALTQHGKEDLKFPRGQGVPINTNSSPDDQIGYYRRATRRIRGGDGKMKDLSPRWYFYYLGTGPEAGLPYGANKDGIIWVATEGALNTPKDHIGTRNPANNAAIVLQLPQGTTLPKGFYAEGSRGGSQASSRSSSRSRNSSRNSTPGSSRGTSPARMAGNGGDAALALLLLDRLNQLESKMSGKGQQQQGQTVTKKSAAEASKKPRQKRTATKAYNVTQAFGRRGPEQTQGNFGDQELIRQGTDYKHWPQIAQFAPSASAFFGMSRIGMEVTPSGTWLTYTGAIKLDDKDPNFKDQVILLNKHIDAYKTFPPTEPKKDKKKKADETQALPQRQKKQQTVTLLPAADLDDFSKQLQQSMSSADSTQA

SEQ ID NO: 4 - DNA, 3822 bp, synthetic construct
  source 1..3822: mol_type = other DNA
  misc_feature 1..3822: note = S nucleotide sequence (Wuhan-Hu-1 strain). NCBI NC045512.2. Gene ID: 43740568). 3822 bp
atgtttgtttttcttgttttattgccactagtctctagtcagtgtgttaatcttacaaccagaactcaattaccccctgcatacactaattctttcacacgtggtgtttattaccctgacaaagttttcagatcctcagttttacattcaactcaggacttgttcttacctttcttttccaatgttacttggttccatgctatacatgtctctgggaccaatggtactaagaggtttgataaccctgtcctaccatttaatgatggtgtttattttgcttccactgagaagtctaacataataagaggctggatttttggtactactttagattcgaagacccagtccctacttattgttaataacgctactaatgttgttattaaagtctgtgaatttcaattttgtaatgatccatttttgggtgtttattaccacaaaaacaacaaaagttggatggaaagtgagttcagagtttattctagtgcgaataattgcacttttgaatatgtctctcagccttttcttatggaccttgaaggaaaacagggtaatttcaaaaatcttagggaatttgtgtttaagaatattgatggttattttaaaatatattctaagcacacgcctattaatttagtgcgtgatctccctcagggtttttcggctttagaaccattggtagatttgccaataggtattaacatcactaggtttcaaactttacttgctttacatagaagttatttgactcctggtgattcttcttcaggttggacagctggtgctgcagcttattatgtgggttatcttcaacctaggacttttctattaaaatataatgaaaatggaaccattacagatgctgtagactgtgcacttgaccctctctcagaaacaaagtgtacgttgaaatccttcactgtagaaaaaggaatctatcaaacttctaactttagagtccaaccaacagaatctattgttagatttcctaatattacaaacttgtgcccttttggtgaagtttttaacgccaccagatttgcatctgtttatgcttggaacaggaagagaatcagcaactgtgttgctgattattctgtcctatataattccgcatcattttccacttttaagtgttatggagtgtctcctactaaattaaatgatctctgctttactaatgtctatgcagattcatttgtaattagaggtgatgaagtcagacaaatcgctccagggcaaactggaaagattgctgattataattataaattaccagatgattttacaggctgcgttatagcttggaattctaacaatcttgattctaaggttggtggtaattataattacctgtatagattgtttaggaagtctaatctcaaaccttttgagagagatatttcaactgaaatctatcaggccggtagcacaccttgtaatggtgttgaaggttttaattgttactttcctttacaatcatatggtttccaacccactaatggtgttggttaccaaccatacagagtagtagtactttcttttgaacttctacatgcaccagcaactgtttgtggacctaaaaagtctactaatttggttaaaaacaaatgtgtcaatttcaacttcaatggtttaacaggcacaggtgttcttactgagtctaacaaaaagtttctgcctttccaacaatttggcagagacattgctgacactactgatgctgtccgtgatccacagacacttgagattcttgacattacaccatgttcttttggtggtgtcagtgttataacaccaggaacaaatacttctaaccaggttgctgttctttatcaggatgttaactgcacagaagtccctgttgctattcatgcagatcaacttactcctacttggcgtgtttattctacaggttctaatgtttttcaaacacgtgcaggctgtttaataggggctgaacatgtcaacaactcatatgagtgtgacatacccattggtgcaggtatatgcgctagttatcagactcagactaattctcctcggcgggcacgtagtgtagctagtcaatccatcattgcctacactatgtcacttggtgcagaaaattcagttgcttactctaataactctattgccatacccacaaattttactattagtgttaccacagaaattctaccagtgtctatgaccaagacatcagtagattgtacaatgtacatttgtggtgattcaactgaatgcagcaatcttttgttgcaatatggcagtttttgtacacaattaaaccgtgctttaactggaatagctgttgaacaagacaaaaacacccaagaagtttttgcacaagtcaaacaaatttacaaaacaccaccaattaaagattttggtggttttaatttttcacaaatattaccagatccatcaaaaccaagcaagaggtcatttattgaagatctacttttcaacaaagtgacacttgcagatgctggcttcatcaaacaatatggtgattgccttggtgatattgctgctagagacctcatttgtgcacaaaagtttaacggccttactgttttgccacctttgctcacagatgaaatgattgctcaatacacttctgcactgttagcgggtacaatcacttctggttggacctttggtgcaggtgctgcattacaaataccatttgctatgcaaatggcttataggtttaatggtattggagttacacagaatgttctctatgagaaccaaaaattgattgccaaccaatttaatagtgctattggcaaaattcaagactcactttcttccacagcaagtgcacttggaaaacttcaagatgtggtcaaccaaaatgcacaagctttaaacacgcttgttaaacaacttagctccaattttggtgcaatttcaagtgttttaaatgatatcctttcacgtcttgacaaagttgaggctgaagtgcaaattgataggttgatcacaggcagacttcaaagtttgcagacatatgtgactcaacaattaattagagctgcagaaatcagagcttctgctaatcttgctgctactaaaatgtcagagtgtgtacttggacaatcaaaaagagttgatttttgtggaaagggctatcatcttatgtccttccctcagtcagcacctcatggtgtagtcttcttgcatgtgacttatgtccctgcacaagaaaagaacttcacaactgctcctgccatttgtcatgatggaaaagcacactttcctcgtgaaggtgtctttgtttcaaatggcacacactggtttgtaacacaaaggaatttttatgaaccacaaatcattactacagacaacacatttgtgtctggtaactgtgatgttgtaataggaattgtcaacaacacagtttatgatcctttgcaacctgaattagactcattcaaggaggagttagataaatattttaagaatcatacatcaccagatgttgatttaggtgacatctctggcattaatgcttcagttgtaaacattcaaaaagaaattgaccgcctcaatgaggttgccaagaatttaaatgaatctctcatcgatctccaagaacttggaaagtatgagcagtatataaaatggccatggtacatttggctaggttttatagctggcttgattgccatagtaatggtgacaattatgctttgctgtatgaccagttgctgtagttgtctcaagggctgttgttcttgtggatcctgctgcaaatttgatgaagacgactctgagccagtgctcaaaggagtcaaattacattacacataa

SEQ ID NO: 5 - DNA, 3815 bp, synthetic construct
  source 1..3815: mol_type = other DNA
  misc_feature 1..3815: note = Codon-optimized for expression in human S nucleotide sequence
atgttcgtttttctggtgctgctccccctcgtgtctagccagtgcgtcaacctcacaacacgcacccagctgccacccgcctacactaattctttcacaagaggggtctattaccccgataaggtgtttcggtctagcgtgctgcattccacccaagacctcttcctgcccttctttagcaacgtgacttggtttcacgccattcatgtgtccggaacaaatgggactaaacggtttgataaccccgttctgcctttcaatgacggcgtgtactttgcaagcaccgagaagagcaatatcattagggggtggatttttggcacaaccctcgattccaagacacaaagcctgctgatcgtgaacaacgcaactaatgtggtgatcaaggtctgcgaattccaattctgtaatgacccatttctcggcgtctactatcacaagaacaacaagagctggatggaatccgaatttcgcgtctattcttccgcaaataactgcactttcgaatatgtgtctcagccattcctcatggacctcgagggaaaacagggcaacttcaaaaatctgagggagttcgtcttcaagaacattgatgggtacttcaagatttacagcaagcatacccccatcaacctggtccgggatctcccacagggcttctccgcactcgaacctctggtggacctccctatcgggattaatatcacaagatttcagactctgctggccctgcacaggtcttatctcaccccaggggattcttcttccggatggacagccggagccgccgcttattacgttggatacctgcagcctaggacctttctgctgaaatacaatgagaatgggacaattaccgacgctgtcgattgcgctctggatcccctgtctgagaccaaatgcaccctgaaatctttcactgtcgagaagggaatctaccagacttccaattttagggttcagcccaccgaaagcatcgtcaggtttcctaacatcacaaatctgtgtccttttggagaggtgtttaacgctactcgctttgcctctgtttacgcctggaacaggaagcgcattagcaattgtgtggccgattatagcgtgctctacaattctgcttctttctccacattcaaatgctacggcgtgtctcctactaagctcaatgacctgtgttttacaaacgtgtatgccgattccttcgtcatcagaggggatgaagttagacagatcgctccagggcagactggaaaaatcgccgactacaattataagctcccagacgatttcactggctgcgtgatcgcatggaattccaacaatctcgactccaaggtcggcggcaattacaattatctctatagactgttccggaagagcaacctcaagccatttgagagggacatttctaccgagatttaccaagctggatccaccccttgtaacggcgtcgaaggcttcaactgttactttcccctgcagagctacggattccagccaaccaatggcgtgggctatcaaccctatagagtcgtggtgctcagcttcgaactgctccacgcccccgcaaccgtctgtggacccaaaaagagcaccaacctggtcaagaacaaatgcgtgaactttaatttcaacgggctcaccgggacaggcgtgctgacagagagcaataagaaattcctccccttccagcaattcggccgggatatcgccgacacaacagatgctgtgagggacccacagacactggaaatcctcgacattacaccctgcagctttgggggcgttagcgtgattacaccaggaacaaatacaagcaaccaggttgccgtgctgtatcaggatgtgaattgtacagaggtgcccgtggcaatccacgccgaccagctcacaccaacctggcgcgtctactccactgggagcaacgtctttcagaccagggccgggtgcctgatcggagctgagcacgtcaacaattcttacgaatgcgatatccccattggggccggaatctgcgcatcctatcagacccaaacaaacagcccacggcgcgctcggtctgtggcttcccagagcatcatcgcttacaccatgagcctcggcgctgagaattccgtcgcttatagcaacaattccatcgccatcccaactaatttcacaatctccgttaccacagagatcctgcctgtttctatgaccaagacttccgtggactgtaccatgtatatttgtggagatagcaccgaatgtagcaacctgctgctgcaatatggctccttttgcacccagctgaacagagcactgactgggattgccgttgagcaggataagaatacccaggaggtttttgctcaggtgaaacagatttacaagaccccacccattaaagactttgggggattcaactttagccagattctccctgacccttccaaaccctccaaacgcagctttattgaagatctgctgttcaacaaggtgaccctggcagatgcaggcttcatcaaacaatatggggactgcctgggagacattgctgcccgcgacctgatctgcgcccagaaatttaacggcctcaccgtcctgcccccactgctgacagacgagatgattgcccaatacactagcgccctgctggcaggcactattacttctggctggacattcggagccggcgccgccctccaaatccctttcgctatgcagatggcctatcggttcaacggcatcggggtgactcagaacgttctgtacgagaaccagaaactgattgccaaccaattcaacagcgcaattggcaagatccaagactccctgagctctacagcctccgccctcgggaaactccaggacgtggttaaccagaatgcccaggcactgaacaccctggtgaaacagctgtccagcaattttggcgcaatctcctccgtgctgaacgacattctgtctcgcctggacaaggttgaagctgaggtgcagattgatagactgatcactggacgcctgcaaagcctgcagacatacgtcactcagcagctgatcagggcagccgaaatcagagcctccgcaaacctggctgcaactaagatgtctgaatgcgtcctgggccaatccaagcgggtggatttttgcggaaaggggtatcacctgatgagcttccctcagagcgctccacatggcgtggtgtttctccacgtgacctacgtgcctgctcaagagaaaaatttcactaccgcacctgccatctgccacgatggaaaggcacattttccaagagagggcgtgttcgtcagcaatggcactcattggtttgtgacccagcggaacttttatgaacctcagatcatcaccaccgataatactttcgtgtccggcaactgtgacgtggttattgggatcgtcaataataccgtctatgatcctctccagcccgagctcgactcctttaaagaggaactggacaagtacttcaagaatcacacttctcctgatgtggatctgggagatatctctggcattaacgcttctgttgtgaacattcagaaggagatcgacagactgaatgaggttgccaaaaatctgaacgaatccctcatcgacctgcaggaactggggaagtacgagcaatatattaaatggccttggtacatttggctcggattcattgctggcctgatcgctatcgttatggtgaccattatgctgtgctgtatgacatcttgttgtagctgtctgaaagggtgctgctcttgcggatcttgttgtaaatttgacgaggatgactctgagcccgttctgaagggggtgaagctccatta

SEQ ID NO: 6 - DNA, 3822 bp, synthetic construct
  source 1..3822: mol_type = other DNA
  misc_feature 1..3822: note = codon-optimized for expression in human S nucleotide sequence with a modification in the sequence encoding the furin cleavage site (Sfs)
atgttcgtttttctggtgctgctccccctcgtgtctagccagtgcgtcaacctcacaacacgcacccagctgccacccgcctacactaattctttcacaagaggggtctattaccccgataaggtgtttcggtctagcgtgctgcattccacccaagacctcttcctgcccttctttagcaacgtgacttggtttcacgccattcatgtgtccggaacaaatgggactaaacggtttgataaccccgttctgcctttcaatgacggcgtgtactttgcaagcaccgagaagagcaatatcattagggggtggatttttggcacaaccctcgattccaagacacaaagcctgctgatcgtgaacaacgcaactaatgtggtgatcaaggtctgcgaattccaattctgtaatgacccatttctcggcgtctactatcacaagaacaacaagagctggatggaatccgaatttcgcgtctattcttccgcaaataactgcactttcgaatatgtgtctcagccattcctcatggacctcgagggaaaacagggcaacttcaaaaatctgagggagttcgtcttcaagaacattgatgggtacttcaagatttacagcaagcatacccccatcaacctggtccgggatctcccacagggcttctccgcactcgaacctctggtggacctccctatcgggattaatatcacaagatttcagactctgctggccctgcacaggtcttatctcaccccaggggattcttcttccggatggacagccggagccgccgcttattacgttggatacctgcagcctaggacctttctgctgaaatacaatgagaatgggacaattaccgacgctgtcgattgcgctctggatcccctgtctgagaccaaatgcaccctgaaatctttcactgtcgagaagggaatctaccagacttccaattttagggttcagcccaccgaaagcatcgtcaggtttcctaacatcacaaatctgtgtccttttggagaggtgtttaacgctactcgctttgcctctgtttacgcctggaacaggaagcgcattagcaattgtgtggccgattatagcgtgctctacaattctgcttctttctccacattcaaatgctacggcgtgtctcctactaagctcaatgacctgtgttttacaaacgtgtatgccgattccttcgtcatcagaggggatgaagttagacagatcgctccagggcagactggaaaaatcgccgactacaattataagctcccagacgatttcactggctgcgtgatcgcatggaattccaacaatctcgactccaaggtcggcggcaattacaattatctctatagactgttccggaagagcaacctcaagccatttgagagggacatttctaccgagatttaccaagctggatccaccccttgtaacggcgtcgaaggcttcaactgttactttcccctgcagagctacggattccagccaaccaatggcgtgggctatcaaccctatagagtcgtggtgctcagcttcgaactgctccacgcccccgcaaccgtctgtggacccaaaaagagcaccaacctggtcaagaacaaatgcgtgaactttaatttcaacgggctcaccgggacaggcgtgctgacagagagcaataagaaattcctccccttccagcaattcggccgggatatcgccgacacaacagatgctgtgagggacccacagacactggaaatcctcgacattacaccctgcagctttgggggcgttagcgtgattacaccaggaacaaatacaagcaaccaggttgccgtgctgtatcaggatgtgaattgtacagaggtgcccgtggcaatccacgccgaccagctcacaccaacctggcgcgtctactccactgggagcaacgtctttcagaccagggccgggtgcctgatcggagctgagcacgtcaacaattcttacgaatgcgatatccccattggggccggaatctgcgcatcctatcagacccaaacaaacagcccaggcggcagcggctctgtggcttcccagagcatcatcgcttacaccatgagcctcggcgctgagaattccgtcgcttatagcaacaattccatcgccatcccaactaatttcacaatctccgttaccacagagatcctgcctgtttctatgaccaagacttccgtggactgtaccatgtatatttgtggagatagcaccgaatgtagcaacctgctgctgcaatatggctccttttgcacccagctgaacagagcactgactgggattgccgttgagcaggataagaatacccaggaggtttttgctcaggtgaaacagatttacaagaccccacccattaaagactttgggggattcaactttagccagattctccctgacccttccaaaccctccaaacgcagctttattgaagatctgctgttcaacaaggtgaccctggcagatgcaggcttcatcaaacaatatggggactgcctgggagacattgctgcccgcgacctgatctgcgcccagaaatttaacggcctcaccgtcctgcccccactgctgacagacgagatgattgcccaatacactagcgccctgctggcaggcactattacttctggctggacattcggagccggcgccgccctccaaatccctttcgctatgcagatggcctatcggttcaacggcatcggggtgactcagaacgttctgtacgagaaccagaaactgattgccaaccaattcaacagcgcaattggcaagatccaagactccctgagctctacagcctccgccctcgggaaactccaggacgtggttaaccagaatgcccaggcactgaacaccctggtgaaacagctgtccagcaattttggcgcaatctcctccgtgctgaacgacattctgtctcgcctggacaaggttgaagctgaggtgcagattgatagactgatcactggacgcctgcaaagcctgcagacatacgtcactcagcagctgatcagggcagccgaaatcagagcctccgcaaacctggctgcaactaagatgtctgaatgcgtcctgggccaatccaagcgggtggatttttgcggaaaggggtatcacctgatgagcttccctcagagcgctccacatggcgtggtgtttctccacgtgacctacgtgcctgctcaagagaaaaatttcactaccgcacctgccatctgccacgatggaaaggcacattttccaagagagggcgtgttcgtcagcaatggcactcattggtttgtgacccagcggaacttttatgaacctcagatcatcaccaccgataatactttcgtgtccggcaactgtgacgtggttattgggatcgtcaataataccgtctatgatcctctccagcccgagctcgactcctttaaagaggaactggacaagtacttcaagaatcacacttctcctgatgtggatctgggagatatctctggcattaacgcttctgttgtgaacattcagaaggagatcgacagactgaatgaggttgccaaaaatctgaacgaatccctcatcgacctgcaggaactggggaagtacgagcaatatattaaatggccttggtacatttggctcggattcattgctggcctgatcgctatcgttatggtgaccattatgctgtgctgtatgacatcttgttgtagctgtctgaaagggtgctgctcttgcggatcttgttgtaaatttgacgaggatgactctgagcccgttctgaagggggtgaagctccattacacctga

SEQ ID NO: 7 - DNA, 1260 bp, synthetic construct
  source 1..1260: mol_type = other DNA
  misc_feature 1..1260: note = N nucleotide sequence (Wuhan-Hu-1 strain). NCBI NC045512.2. Gene ID: 43740575
atgtctgataatggaccccaaaatcagcgaaatgcaccccgcattacgtttggtggaccctcagattcaactggcagtaaccagaatggagaacgcagtggggcgcgatcaaaacaacgtcggccccaaggtttacccaataatactgcgtcttggttcaccgctctcactcaacatggcaaggaagaccttaaattccctcgaggacaaggcgttccaattaacaccaatagcagtccagatgaccaaattggctactaccgaagagctaccagacgaattcgtggtggtgacggtaaaatgaaagatctcagtccaagatggtatttctactacctaggaactgggccagaagctggacttccctatggtgctaacaaagacggcatcatatgggttgcaactgagggagccttgaatacaccaaaagatcacattggcacccgcaatcctgctaacaatgctgcaatcgtgctacaacttcctcaaggaacaacattgccaaaaggcttctacgcagaagggagcagaggcggcagtcaagcctcttctcgttcctcatcacgtagtcgcaacagttcaagaaattcaactccaggcagcagtaggggaacttctcctgctagaatggctggcaatggcggtgatgctgctcttgctttgctgctgcttgacagattgaaccagcttgagagcaaaatgtctggtaaaggccaacaacaacaaggccaaactgtcactaagaaatctgctgctgaggcttctaagaagcctcggcaaaaacgtactgccactaaagcatacaatgtaacacaagctttcggcagacgtggtccagaacaaacccaaggaaattttggggaccaggaactaatcagacaaggaactgattacaaacattggccgcaaattgcacaatttgcccccagcgcttcagcgttcttcggaatgtcgcgcattggcatggaagtcacaccttcgggaacgtggttgacctacacaggtgccatcaaattggatgacaaagatccaaatttcaaagatcaagtcattttgctgaataagcatattgacgcatacaaaacattcccaccaacagagcctaaaaaggacaaaaagaagaaggctgatgaaactcaagccttaccgcagagacagaagaaacagcaaactgtgactcttcttcctgctgcagatttggatgatttctccaaacaattgcaacaatccatgagcagtgctgactcaactcaggcctaa

SEQ ID NO: 8 - DNA, 1260 bp, synthetic construct
  source 1..1260: mol_type = other DNA
  misc_feature 1..1260: note = codon-optimized for human expression N nucleotide sequence
atgtccgataacggcccccagaaccaacgcaatgcccctcggattacattcggcggacccagcgactccaccgggagcaaccaaaacggcgagcgcagcggagcacggtctaagcagagaaggcctcaggggctgccaaataacactgcttcttggttcactgctctgacacagcatggaaaagaggacctcaaatttccccggggccagggcgttcccatcaacactaactcttccccagatgaccagatcgggtattaccgcagggctactcggagaatcaggggcggggacgggaaaatgaaggatctcagcccaaggtggtacttttattatctcggcacagggcctgaagccggactgccctatggagctaacaaagacggcattatttgggtggcaactgagggcgccctgaacaccccaaaagatcatatcggaacccgcaatcctgccaataacgctgccattgtgctccagctgcctcaggggacaacactgcccaaagggttctacgcagaaggcagccgcgggggatctcaggcaagctctcggtcctcttctagatccagaaacagctctaggaattccaccccagggtcctccagaggaacatccccagctagaatggcaggaaatggaggcgacgctgcactggcactgctgctgctggacagactgaaccagctcgagagcaaaatgtctggaaaggggcagcagcagcaagggcagaccgtcaccaagaagagcgccgccgaagctagcaagaaacctaggcagaaaaggaccgcaacaaaggcctataatgtgacccaagccttcggacgccgcggcccagaacagacccaaggcaatttcggcgaccaggagctgatccggcaaggcactgattacaagcactggccacagattgctcaattcgcccccagcgctagcgccttctttggaatgtcccggattggcatggaggtgacaccatctggcacttggctcacctacacaggggctatcaagctcgatgacaaagatcccaattttaaagaccaggtcatcctgctgaataaacacatcgatgcatacaagacttttcctcctactgaacccaaaaaggataagaagaagaaagcagatgagacccaggccctgccccagagacaaaagaagcagcagaccgttacactgctccctgccgccgacctcgacgatttttccaagcagctgcagcaatctatgagcagcgccgactccacccaggcctag

SEQ ID NO: 9 - DNA, 7722 bp, synthetic construct
  source 1..7722: mol_type = other DNA
  misc_feature 1..7722: note = pPAL-S
ggtaccatgtttgtttttcttgttttattgccactagtctctagtcagtgtgttaatcttacaaccagaactcaattaccccctgcatacactaattctttcacacgtggtgtttattaccctgacaaagttttcagatcctcagttttacattcaactcaggacttgttcttacctttcttttccaatgttacttggttccatgctatacatgtctctgggaccaatggtactaagaggtttgataaccctgtcctaccatttaatgatggtgtttattttgcttccactgagaagtctaacataataagaggctggatttttggtactactttagattcgaagacccagtccctacttattgttaataacgctactaatgttgttattaaagtctgtgaatttcaattttgtaatgatccatttttgggtgtttattaccacaaaaacaacaaaagttggatggaaagtgagttcagagtttattctagtgcgaataattgcacttttgaatatgtctctcagccttttcttatggaccttgaaggaaaacagggtaatttcaaaaatcttagggaatttgtgtttaagaatattgatggttattttaaaatatattctaagcacacgcctattaatttagtgcgtgatctccctcagggtttttcggctttagaaccattggtagatttgccaataggtattaacatcactaggtttcaaactttacttgctttacatagaagttatttgactcctggtgattcttcttcaggttggacagctggtgctgcagcttattatgtgggttatcttcaacctaggacttttctattaaaatataatgaaaatggaaccattacagatgctgtagactgtgcacttgaccctctctcagaaacaaagtgtacgttgaaatccttcactgtagaaaaaggaatctatcaaacttctaactttagagtccaaccaacagaatctattgttagatttcctaatattacaaacttgtgcccttttggtgaagtttttaacgccaccagatttgcatctgtttatgcttggaacaggaagagaatcagcaactgtgttgctgattattctgtcctatataattccgcatcattttccacttttaagtgttatggagtgtctcctactaaattaaatgatctctgctttactaatgtctatgcagattcatttgtaattagaggtgatgaagtcagacaaatcgctccagggcaaactggaaagattgctgattataattataaattaccagatgattttacaggctgcgttatagcttggaattctaacaatcttgattctaaggttggtggtaattataattacctgtatagattgtttaggaagtctaatctcaaaccttttgagagagatatttcaactgaaatctatcaggccggtagcacaccttgtaatggtgttgaaggttttaattgttactttcctttacaatcatatggtttccaacccactaatggtgttggttaccaaccatacagagtagtagtactttcttttgaacttctacatgcaccagcaactgtttgtggacctaaaaagtctactaatttggttaaaaacaaatgtgtcaatttcaacttcaatggtttaacaggcacaggtgttcttactgagtctaacaaaaagtttctgcctttccaacaatttggcagagacattgctgacactactgatgctgtccgtgatccacagacacttgagattcttgacattacaccatgttcttttggtggtgtcagtgttataacaccaggaacaaatacttctaaccaggttgctgttctttatcaggatgttaactgcacagaagtccctgttgctattcatgcagatcaacttactcctacttggcgtgtttattctacaggttctaatgtttttcaaacacgtgcaggctgtttaataggggctgaacatgtcaacaactcatatgagtgtgacatacccattggtgcaggtatatgcgctagttatcagactcagactaattctcctcggcgggcacgtagtgtagctagtcaatccatcattgcctacactatgtcacttggtgcagaaaattcagttgcttactctaataactctattgccatacccacaaattttactattagtgttaccacagaaattctaccagtgtctatgaccaagacatcagtagattgtacaatgtacatttgtggtgattcaactgaatgcagcaatcttttgttgcaatatggcagtttttgtacacaattaaaccgtgctttaactggaatagctgttgaacaagacaaaaacacccaagaagtttttgcacaagtcaaacaaatttacaaaacaccaccaattaaagattttggtggttttaatttttcacaaatattaccagatccatcaaaaccaagcaagaggtcatttattgaagatctacttttcaacaaagtgacacttgcagatgctggcttcatcaaacaatatggtgattgccttggtgatattgctgctagagacctcatttgtgcacaaaagtttaacggccttactgttttgccacctttgctcacagatgaaatgattgctcaatacacttctgcactgttagcgggtacaatcacttctggttggacctttggtgcaggtgctgcattacaaataccatttgctatgcaaatggcttataggtttaatggtattggagttacacagaatgttctctatgagaaccaaaaattgattgccaaccaatttaatagtgctattggcaaaattcaagactcactttcttccacagcaagtgcacttggaaaacttcaagatgtggtcaaccaaaatgcacaagctttaaacacgcttgttaaacaacttagctccaattttggtgcaatttcaagtgttttaaatgatatcctttcacgtcttgacaaagttgaggctgaagtgcaaattgataggttgatcacaggcagacttcaaagtttgcagacatatgtgactcaacaattaattagagctgcagaaatcagagcttctgctaatcttgctgctactaaaatgtcagagtgtgtacttggacaatcaaaaagagttgatttttgtggaaagggctatcatcttatgtccttccctcagtcagcacctcatggtgtagtcttcttgcatgtgacttatgtccctgcacaagaaaagaacttcacaactgctcctgccatttgtcatgatggaaaagcacactttcctcgtgaaggtgtctttgtttcaaatggcacacactggtttgtaacacaaaggaatttttatgaaccacaaatcattactacagacaacacatttgtgtctggtaactgtgatgttgtaataggaattgtcaacaacacagtttatgatcctttgcaacctgaattagactcattcaaggaggagttagataaatattttaagaatcatacatcaccagatgttgatttaggtgacatctctggcattaatgcttcagttgtaaacattcaaaaagaaattgaccgcctcaatgaggttgccaagaatttaaatgaatctctcatcgatctccaagaacttggaaagtatgagcagtatataaaatggccatggtacatttggctaggttttatagctggcttgattgccatagtaatggtgacaattatgctttgctgtatgaccagttgctgtagttgtctcaagggctgttgttcttgtggatcctgctgcaaatttgatgaagacgactctgagccagtgctcaaaggagtcaaattacattacacataatctagagtcgacccgggcggccgcttccctttagtgagggttaatgcttcgagcagacatgataagatacattgatgagtttggacaaaccacaactagaatgcagtgaaaaaaatgctttatttgtgaaatttgtgatgctattgctttatttgtaaccattataagctgcaataaacaagttaacaacaacaattgcattcattttatgtttcaggttcagggggagatgtgggaggttttttaaagcaagtaaaacctctacaaatgtggtaaaatccgataaggatcgatccgggctggcgtaatagcgaagaggcccgcaccgatcgcccttcccaacagttgcgcagcctgaatggcgaatggacgcgccctgtagcggcgcattaagcgcggcgggtgtggtggttacgcgcagcgtgaccgctacacttgccagcgttaattaagtgctggagaatattcggcaaggtctgaaccgtcccagccatcgccatgaaagggttaggggctgtatgagcctgtttgttgctggggtaacaatatttgcacaatacggtcccctcgcccctctggggagagggttagggtgaggggaaaagcgccccccctgccgcagcctgctccggtcggacctggcaactatagctactcacagccaggttgattataataaccgtttatctgttcgtactgtttactaaaacgacgaatcgcctgattttcaggcacaacaagcatcaacaataaggattaaagctatgggttttctttccggtaagcgcattctggtaaccggtgttgccagcaaactatccatcgcctacggtatcgctcaggcgatgcaccgcgaaggagctgaactggcattcacctaccagaacgacaaactgaaaggccgcgtagaagaatttgccgctcaattgggttctgacatcgttctgcagtgcgatgttgcagaagatgccagcatcgacaccatgttcgctgaactggggaaagtttggccgaaatttgacggtttcgtacactctattggttttgcacctggcgatcagctggatggtgactatgttaacgccgttacccgtgaaggcttcaaaattgcccacgacatcagctcctacagcttcgttgcaatggcaaaagcttgccgctccatgctgaatccgggttctgccctgctgaccctttcctaccttggcgctgagcgcgctatcccgaactacaacgttatgggtctggcaaaagcgtctctggaagcgaacgtgcgctatatggcgaacgcgatgggtccggaaggtgtgcgtgttaacgccatctctgctggtccgatccgtactctggcggcttccggtatcaaagacttccgcaaaatgctggctcattgcgaagccgttaccccgattcgccgtaccgttactattgaagatgtgggtaactctgcggcattcctgtgctccgatctctctgccggtatctccggtgaagtagtccacgttgacggcggtttcagcatcgctgcaatgaacgaactcgaactgaaataattaattaaccgcgtatggtgcactctcagtacaatctgctctgatgccgcatagttaagccagccccgacacccgccaacacccgctgacgcgccctgacgggcttgtctgctcccggcatccgcttacagacaagctgtgaccgtctccgggagctcatgtgtcagaggttttcacaagttgcaggaccacttctgcgctcggcccttccggctggctggtttattgctgataaatctggagccggtgagcgtgggtctcgcggtatcattgcagcactggggccagatggtaagccctcccgtatcgtagttatctacacgacggggagtcaggcaactatggatgaacgaaatagacagatcgctgagataggtgcctcactgattaagcattggtaactgtcagaccaagtttactcatatatactttagattgatttaaaacttcatttttaatttaaaaggatctaggtgaagatcctttttgataatctcatgaccaaaatcccttaacgtgagttttcgttccactgagcgtcagaccccgtagaaaagatcaaaggatcttcttgagatcctttttttctgcgcgtaatctgctgcttgcaaacaaaaaaaccaccgctaccagcggtggtttgtttgccggatcaagagctaccaactctttttccgaaggtaactggcttcagcagagcgcagataccaaatactgtccttctagtgtagccgtagttaggccaccacttcaagaactctgtagcaccgcctacatacctcgctctgctaatcctgttaccagtggctgctgccagtggcgataagtcgtgtcttaccgggttggactcaagacgatagttaccggataaggcgcagcggtcgggctgaacggggggttcgtgcacacagcccagcttggagcgaacgacctacaccgaactgagatacctacagcgtgagctatgagaaagcgccacgcttcccgaagggagaaaggcggacaggtatccggtaagcggcagggtcggaacaggagagcgcacgagggagcttccagggggaaacgcctggtatctttatagtcctgtcgggtttcgccacctctgacttgagcgtcgatttttgtgatgctcgtcaggggggcggagcctatggaaaaacgccagcaacgcggcctttttacggttcctggccttttgctggccttttgctcacatggctcgacagatcttcaatattggccattagccatattattcattggttatatagcataaatcaatattggctattggccattgcatacgttgtatctatatcataatatgtacatttatattggctcatgtccaatatgaccgccatgttggcattgattattgactagttattaatagtaatcaattacggggtcattagttcatagcccatatatggagttccgcgttacataacttacggtaaatggcccgcctggctgaccgcccaacgacccccgcccattgacgtcaataatgacgtatgttcccatagtaacgccaatagggactttccattgacgtcaatgggtggagtatttacggtaaactgcccacttggcagtacatcaagtgtatcatatgccaagtccgccccctattgacgtcaatgacggtaaatggcccgcctggcattatgcccagtacatgaccttacgggactttcctacttggcagtacatctacgtattagtcatcgctattaccatggtgatgcggttttggcagtacaccaatgggcgtggatagcggtttgactcacggggatttccaagtctccaccccattgacgtcaatgggagtttgttttggcaccaaaatcaacgggactttccaaaatgtcgtaacaactgcgatcgcccgccccgttgacgcaaatgggcggtaggcgtgtacggtgggaggtctatataagcagagctcgtttagtgaaccgtcagatcactagaagctttattgcggtagtttatcacagttaaattgctaacgcagtcagtgcttctgacacaacagtctcgaacttaagctgcagtgactctcttaaggtagccttgcagaagttggtcgtgaggcactgggcaggtaagtatcaaggttacaagacaggtttaaggagaccaatagaaactgggcttgtcgagacagagaagactcttgcgtttctgataggcacctattggtcttactgacatccactttgcctttctctccacaggtgtccactcccagttcaattacagctcttaaggctagagtacttaatacgactcactataggctagcctcgagacgcgtggtacc

SEQ ID NO: 10 - DNA, 7722 bp, synthetic construct
  source 1..7722: mol_type = other DNA
  misc_feature 1..7722: note = pPAL-S (codon-optimized S gene)
ggtaccatgttcgtttttctggtgctgctccccctcgtgtctagccagtgcgtcaacctcacaacacgcacccagctgccacccgcctacactaattctttcacaagaggggtctattaccccgataaggtgtttcggtctagcgtgctgcattccacccaagacctcttcctgcccttctttagcaacgtgacttggtttcacgccattcatgtgtccggaacaaatgggactaaacggtttgataaccccgttctgcctttcaatgacggcgtgtactttgcaagcaccgagaagagcaatatcattagggggtggatttttggcacaaccctcgattccaagacacaaagcctgctgatcgtgaacaacgcaactaatgtggtgatcaaggtctgcgaattccaattctgtaatgacccatttctcggcgtctactatcacaagaacaacaagagctggatggaatccgaatttcgcgtctattcttccgcaaataactgcactttcgaatatgtgtctcagccattcctcatggacctcgagggaaaacagggcaacttcaaaaatctgagggagttcgtcttcaagaacattgatgggtacttcaagatttacagcaagcatacccccatcaacctggtccgggatctcccacagggcttctccgcactcgaacctctggtggacctccctatcgggattaatatcacaagatttcagactctgctggccctgcacaggtcttatctcaccccaggggattcttcttccggatggacagccggagccgccgcttattacgttggatacctgcagcctaggacctttctgctgaaatacaatgagaatgggacaattaccgacgctgtcgattgcgctctggatcccctgtctgagaccaaatgcaccctgaaatctttcactgtcgagaagggaatctaccagacttccaattttagggttcagcccaccgaaagcatcgtcaggtttcctaacatcacaaatctgtgtccttttggagaggtgtttaacgctactcgctttgcctctgtttacgcctggaacaggaagcgcattagcaattgtgtggccgattatagcgtgctctacaattctgcttctttctccacattcaaatgctacggcgtgtctcctactaagctcaatgacctgtgttttacaaacgtgtatgccgattccttcgtcatcagaggggatgaagttagacagatcgctccagggcagactggaaaaatcgccgactacaattataagctcccagacgatttcactggctgcgtgatcgcatggaattccaacaatctcgactccaaggtcggcggcaattacaattatctctatagactgttccggaagagcaacctcaagccatttgagagggacatttctaccgagatttaccaagctggatccaccccttgtaacggcgtcgaaggcttcaactgttactttcccctgcagagctacggattccagccaaccaatggcgtgggctatcaaccctatagagtcgtggtgctcagcttcgaactgctccacgcccccgcaaccgtctgtggacccaaaaagagcaccaacctggtcaagaacaaatgcgtgaactttaatttcaacgggctcaccgggacaggcgtgctgacagagagcaataagaaattcctccccttccagcaattcggccgggatatcgccgacacaacagatgctgtgagggacccacagacactggaaatcctcgacattacaccctgcagctttgggggcgttagcgtgattacaccaggaacaaatacaagcaaccaggttgccgtgctgtatcaggatgtgaattgtacagaggtgcccgtggcaatccacgccgaccagctcacaccaacctggcgcgtctactccactgggagcaacgtctttcagaccagggccgggtgcctgatcggagctgagcacgtcaacaattcttacgaatgcgatatccccattggggccggaatctgcgcatcctatcagacccaaacaaacagcccacggcgcgctcggtctgtggcttcccagagcatcatcgcttacaccatgagcctcggcgctgagaattccgtcgcttatagcaacaattccatcgccatcccaactaatttcacaatctccgttaccacagagatcctgcctgtttctatgaccaagacttccgtggactgtaccatgtatatttgtggagatagcaccgaatgtagcaacctgctgctgcaatatggctccttttgcacccagctgaacagagcactgactgggattgccgttgagcaggataagaatacccaggaggtttttgctcaggtgaaacagatttacaagaccccacccattaaagactttgggggattcaactttagccagattctccctgacccttccaaaccctccaaacgcagctttattgaagatctgctgttcaacaaggtgaccctggcagatgcaggcttcatcaaacaatatggggactgcctgggagacattgctgcccgcgacctgatctgcgcccagaaatttaacggcctcaccgtcctgcccccactgctgacagacgagatgattgcccaatacactagcgccctgctggcaggcactattacttctggctggacattcggagccggcgccgccctccaaatccctttcgctatgcagatggcctatcggttcaacggcatcggggtgactcagaacgttctgtacgagaaccagaaactgattgccaaccaattcaacagcgcaattggcaagatccaagactccctgagctctacagcctccgccctcgggaaactccaggacgtggttaaccagaatgcccaggcactgaacaccctggtgaaacagctgtccagcaattttggcgcaatctcctccgtgctgaacgacattctgtctcgcctggacaaggttgaagctgaggtgcagattgatagactgatcactggacgcctgcaaagcctgcagacatacgtcactcagcagctgatcagggcagccgaaatcagagcctccgcaaacctggctgcaactaagatgtctgaatgcgtcctgggccaatccaagcgggtggatttttgcggaaaggggtatcacctgatgagcttccctcagagcgctccacatggcgtggtgtttctccacgtgacctacgtgcctgctcaagagaaaaatttcactaccgcacctgccatctgccacgatggaaaggcacattttccaagagagggcgtgttcgtcagcaatggcactcattggtttgtgacccagcggaacttttatgaacctcagatcatcaccaccgataatactttcgtgtccggcaactgtgacgtggttattgggatcgtcaataataccgtctatgatcctctccagcccgagctcgactcctttaaagaggaactggacaagtacttcaagaatcacacttctcctgatgtggatctgggagatatctctggcattaacgcttctgttgtgaacattcagaaggagatcgacagactgaatgaggttgccaaaaatctgaacgaatccctcatcgacctgcaggaactggggaagtacgagcaatatattaaatggccttggtacatttggctcggattcattgctggcctgatcgctatcgttatggtgaccattatgctgtgctgtatgacatcttgttgtagctgtctgaaagggtgctgctcttgcggatcttgttgtaaatttgacgaggatgactctgagcccgttctgaagggggtgaagctccattacacctgatctagagtcgacccgggcggccgcttccctttagtgagggttaatgcttcgagcagacatgataagatacattgatgagtttggacaaaccacaactagaatgcagtgaaaaaaatgctttatttgtgaaatttgtgatgctattgctttatttgtaaccattataagctgcaataaacaagttaacaacaacaattgcattcattttatgtttcaggttcagggggagatgtgggaggttttttaaagcaagtaaaacctctacaaatgtggtaaaatccgataaggatcgatccgggctggcgtaatagcgaagaggcccgcaccgatcgcccttcccaacagttgcgcagcctgaatggcgaatggacgcgccctgtagcggcgcattaagcgcggcgggtgtggtggttacgcgcagcgtgaccgctacacttgccagcgttaattaagtgctggagaatattcggcaaggtctgaaccgtcccagccatcgccatgaaagggttaggggctgtatgagcctgtttgttgctggggtaacaatatttgcacaatacggtcccctcgcccctctggggagagggttagggtgaggggaaaagcgccccccctgccgcagcctgctccggtcggacctggcaactatagctactcacagccaggttgattataataaccgtttatctgttcgtactgtttactaaaacgacgaatcgcctgattttcaggcacaacaagcatcaacaataaggattaaagctatgggttttctttccggtaagcgcattctggtaaccggtgttgccagcaaactatccatcgcctacggtatcgctcaggcgatgcaccgcgaaggagctgaactggcattcacctaccagaacgacaaactgaaaggccgcgtagaagaatttgccgctcaattgggttctgacatcgttctgcagtgcgatgttgcagaagatgccagcatcgacaccatgttcgctgaactggggaaagtttggccgaaatttgacggtttcgtacactctattggttttgcacctggcgatcagctggatggtgactatgttaacgccgttacccgtgaaggcttcaaaattgcccacgacatcagctcctacagcttcgttgcaatggcaaaagcttgccgctccatgctgaatccgggttctgccctgctgaccctttcctaccttggcgctgagcgcgctatcccgaactacaacgttatgggtctggcaaaagcgtctctggaagcgaacgtgcgctatatggcgaacgcgatgggtccggaaggtgtgcgtgttaacgccatctctgctggtccgatccgtactctggcggcttccggtatcaaagacttccgcaaaatgctggctcattgcgaagccgttaccccgattcgccgtaccgttactattgaagatgtgggtaactctgcggcattcctgtgctccgatctctctgccggtatctccggtgaagtagtccacgttgacggcggtttcagcatcgctgcaatgaacgaactcgaactgaaataattaattaaccgcgtatggtgcactctcagtacaatctgctctgatgccgcatagttaagccagccccgacacccgccaacacccgctgacgcgccctgacgggcttgtctgctcccggcatccgcttacagacaagctgtgaccgtctccgggagctcatgtgtcagaggttttcacaagttgcaggaccacttctgcgctcggcccttccggctggctggtttattgctgataaatctggagccggtgagcgtgggtctcgcggtatcattgcagcactggggccagatggtaagccctcccgtatcgtagttatctacacgacggggagtcaggcaactatggatgaacgaaatagacagatcgctgagataggtgcctcactgattaagcattggtaactgtcagaccaagtttactcatatatactttagattgatttaaaacttcatttttaatttaaaaggatctaggtgaagatcctttttgataatctcatgaccaaaatcccttaacgtgagttttcgttccactgagcgtcagaccccgtagaaaagatcaaaggatcttcttgagatcctttttttctgcgcgtaatctgctgcttgcaaacaaaaaaaccaccgctaccagcggtggtttgtttgccggatcaagagctaccaactctttttccgaaggtaactggcttcagcagagcgcagataccaaatactgtccttctagtgtagccgtagttaggccaccacttcaagaactctgtagcaccgcctacatacctcgctctgctaatcctgttaccagtggctgctgccagtggcgataagtcgtgtcttaccgggttggactcaagacgatagttaccggataaggcgcagcggtcgggctgaacggggggttcgtgcacacagcccagcttggagcgaacgacctacaccgaactgagatacctacagcgtgagctatgagaaagcgccacgcttcccgaagggagaaaggcggacaggtatccggtaagcggcagggtcggaacaggagagcgcacgagggagcttccagggggaaacgcctggtatctttatagtcctgtcgggtttcgccacctctgacttgagcgtcgatttttgtgatgctcgtcaggggggcggagcctatggaaaaacgccagcaacgcggcctttttacggttcctggccttttgctggccttttgctcacatggctcgacagatcttcaatattggccattagccatattattcattggttatatagcataaatcaatattggctattggccattgcatacgttgtatctatatcataatatgtacatttatattggctcatgtccaatatgaccgccatgttggcattgattattgactagttattaatagtaatcaattacggggtcattagttcatagcccatatatggagttccgcgttacataacttacggtaaatggcccgcctggctgaccgcccaacgacccccgcccattgacgtcaataatgacgtatgttcccatagtaacgccaatagggactttccattgacgtcaatgggtggagtatttacggtaaactgcccacttggcagtacatcaagtgtatcatatgccaagtccgccccctattgacgtcaatgacggtaaatggcccgcctggcattatgcccagtacatgaccttacgggactttcctacttggcagtacatctacgtattagtcatcgctattaccatggtgatgcggttttggcagtacaccaatgggcgtggatagcggtttgactcacggggatttccaagtctccaccccattgacgtcaatgggagtttgttttggcaccaaaatcaacgggactttccaaaatgtcgtaacaactgcgatcgcccgccccgttgacgcaaatgggcggtaggcgtgtacggtgggaggtctatataagcagagctcgtttagtgaaccgtcagatcactagaagctttattgcggtagtttatcacagttaaattgctaacgcagtcagtgcttctgacacaacagtctcgaacttaagctgcagtgactctcttaaggtagccttgcagaagttggtcgtgaggcactgggcaggtaagtatcaaggttacaagacaggtttaaggagaccaatagaaactgggcttgtcgagacagagaagactcttgcgtttctgataggcacctattggtcttactgacatccactttgcctttctctccacaggtgtccactcccagttcaattacagctcttaaggctagagtacttaatacgactcactataggctagcctcgagacgcgtggtacc

SEQ ID NO: 11 - DNA, 7722 bp, synthetic construct
  source 1..7722: mol_type = other DNA
  misc_feature 1..7722: note = pPAL-Sfs (codon-optimized Sfs gene)
ggtaccatgttcgtttttctggtgctgctccccctcgtgtctagccagtgcgtcaacctcacaacacgcacccagctgccacccgcctacactaattctttcacaagaggggtctattaccccgataaggtgtttcggtctagcgtgctgcattccacccaagacctcttcctgcccttctttagcaacgtgacttggtttcacgccattcatgtgtccggaacaaatgggactaaacggtttgataaccccgttctgcctttcaatgacggcgtgtactttgcaagcaccgagaagagcaatatcattagggggtggatttttggcacaaccctcgattccaagacacaaagcctgctgatcgtgaacaacgcaactaatgtggtgatcaaggtctgcgaattccaattctgtaatgacccatttctcggcgtctactatcacaagaacaacaagagctggatggaatccgaatttcgcgtctattcttccgcaaataactgcactttcgaatatgtgtctcagccattcctcatggacctcgagggaaaacagggcaacttcaaaaatctgagggagttcgtcttcaagaacattgatgggtacttcaagatttacagcaagcatacccccatcaacctggtccgggatctcccacagggcttctccgcactcgaacctctggtggacctccctatcgggattaatatcacaagatttcagactctgctggccctgcacaggtcttatctcaccccaggggattcttcttccggatggacagccggagccgccgcttattacgttggatacctgcagcctaggacctttctgctgaaatacaatgagaatgggacaattaccgacgctgtcgattgcgctctggatcccctgtctgagaccaaatgcaccctgaaatctttcactgtcgagaagggaatctaccagacttccaattttagggttcagcccaccgaaagcatcgtcaggtttcctaacatcacaaatctgtgtccttttggagaggtgtttaacgctactcgctttgcctctgtttacgcctggaacaggaagcgcattagcaattgtgtggccgattatagcgtgctctacaattctgcttctttctccacattcaaatgctacggcgtgtctcctactaagctcaatgacctgtgttttacaaacgtgtatgccgattccttcgtcatcagaggggatgaagttagacagatcgctccagggcagactggaaaaatcgccgactacaattataagctcccagacgatttcactggctgcgtgatcgcatggaattccaacaatctcgactccaaggtcggcggcaattacaattatctctatagactgttccggaagagcaacctcaagccatttgagagggacatttctaccgagatttaccaagctggatccaccccttgtaacggcgtcgaaggcttcaactgttactttcccctgcagagctacggattccagccaaccaatggcgtgggctatcaaccctatagagtcgtggtgctcagcttcgaactgctccacgcccccgcaaccgtctgtggacccaaaaagagcaccaacctggtcaagaacaaatgcgtgaactttaatttcaacgggctcaccgggacaggcgtgctgacagagagcaataagaaattcctccccttccagcaattcggccgggatatcgccgacacaacagatgctgtgagggacccacagacactggaaatcctcgacattacaccctgcagctttgggggcgttagcgtgattacaccaggaacaaatacaagcaaccaggttgccgtgctgtatcaggatgtgaattgtacagaggtgcccgtggcaatccacgccgaccagctcacaccaacctggcgcgtctactccactgggagcaacgtctttcagaccagggccgggtgcctgatcggagctgagcacgtcaacaattcttacgaatgcgatatccccattggggccggaatctgcgcatcctatcagacccaaacaaacagcccaggcggcagcggctctgtggcttcccagagcatcatcgcttacaccatgagcctcggcgctgagaattccgtcgcttatagcaacaattccatcgccatcccaactaatttcacaatctccgttaccacagagatcctgcctgtttctatgaccaagacttccgtggactgtaccatgtatatttgtggagatagcaccgaatgtagcaacctgctgctgcaatatggctccttttgcacccagctgaacagagcactgactgggattgccgttgagcaggataagaatacccaggaggtttttgctcaggtgaaacagatttacaagaccccacccattaaagactttgggggattcaactttagccagattctccctgacccttccaaaccctccaaacgcagctttattgaagatctgctgttcaacaaggtgaccctggcagatgcaggcttcatcaaacaatatggggactgcctgggagacattgctgcccgcgacctgatctgcgcccagaaatttaacggcctcaccgtcctgcccccactgctgacagacgagatgattgcccaatacactagcgccctgctggcaggcactattacttctggctggacattcggagccggcgccgccctccaaatccctttcgctatgcagatggcctatcggttcaacggcatcggggtgactcagaacgttctgtacgagaaccagaaactgattgccaaccaattcaacagcgcaattggcaagatccaagactccctgagctctacagcctccgccctcgggaaactccaggacgtggttaaccagaatgcccaggcactgaacaccctggtgaaacagctgtccagcaattttggcgcaatctcctccgtgctgaacgacattctgtctcgcctggacaaggttgaagctgaggtgcagattgatagactgatcactggacgcctgcaaagcctgcagacatacgtcactcagcagctgatcagggcagccgaaatcagagcctccgcaaacctggctgcaactaagatgtctgaatgcgtcctgggccaatccaagcgggtggatttttgcggaaaggggtatcacctgatgagcttccctcagagcgctccacatggcgtggtgtttctccacgtgacctacgtgcctgctcaagagaaaaatttcactaccgcacctgccatctgccacgatggaaaggcacattttccaagagagggcgtgttcgtcagcaatggcactcattggtttgtgacccagcggaacttttatgaacctcagatcatcaccaccgataatactttcgtgtccggcaactgtgacgtggttattgggatcgtcaataataccgtctatgatcctctccagcccgagctcgactcctttaaagaggaactggacaagtacttcaagaatcacacttctcctgatgtggatctgggagatatctctggcattaacgcttctgttgtgaacattcagaaggagatcgacagactgaatgaggttgccaaaaatctgaacgaatccctcatcgacctgcaggaactggggaagtacgagcaatatattaaatggccttggtacatttggctcggattcattgctggcctgatcgctatcgttatggtgaccattatgctgtgctgtatgacatcttgttgtagctgtctgaaagggtgctgctcttgcggatcttgttgtaaatttgacgaggatgactctgagcccgttctgaagggggtgaagctccattacacctgatctagagtcgacccgggcggccgcttccctttagtgagggttaatgcttcgagcagacatgataagatacattgatgagtttggacaaaccacaactagaatgcagtgaaaaaaatgctttatttgtgaaatttgtgatgctattgctttatttgtaaccattataagctgcaataaacaagttaacaacaacaattgcattcattttatgtttcaggttcagggggagatgtgggaggttttttaaagcaagtaaaacctctacaaatgtggtaaaatccgataaggatcgatccgggctggcgtaatagcgaagaggcccgcaccgatcgcccttcccaacagttgcgcagcctgaatggcgaatggacgcgccctgtagcggcgcattaagcgcggcgggtgtggtggttacgcgcagcgtgaccgctacacttgccagcgttaattaagtgctggagaatattcggcaaggtctgaaccgtcccagccatcgccatgaaagggttaggggctgtatgagcctgtttgttgctggggtaacaatatttgcacaatacggtcccctcgcccctctggggagagggttagggtgaggggaaaagcgccccccctgccgcagcctgctccggtcggacctggcaactatagctactcacagccaggttgattataataaccgtttatctgttcgtactgtttactaaaacgacgaatcgcctgattttcaggcacaacaagcatcaacaataaggattaaagctatgggttttctttccggtaagcgcattctggtaaccggtgttgccagcaaactatccatcgcctacggtatcgctcaggcgatgcaccgcgaaggagctgaactggcattcacctaccagaacgacaaactgaaaggccgcgtagaagaatttgccgctcaattgggttctgacatcgttctgcagtgcgatgttgcagaagatgccagcatcgacaccatgttcgctgaactggggaaagtttggccgaaatttgacggtttcgtacactctattggttttgcacctggcgatcagctggatggtgactatgttaacgccgttacccgtgaaggcttcaaaattgcccacgacatcagctcctacagcttcgttgcaatggcaaaagcttgccgctccatgctgaatccgggttctgccctgctgaccctttcctaccttggcgctgagcgcgctatcccgaactacaacgttatgggtctggcaaaagcgtctctggaagcgaacgtgcgctatatggcgaacgcgatgggtccggaaggtgtgcgtgttaacgccatctctgctggtccgatccgtactctggcggcttccggtatcaaagacttccgcaaaatgctggctcattgcgaagccgttaccccgattcgccgtaccgttactattgaagatgtgggtaactctgcggcattcctgtgctccgatctctctgccggtatctccggtgaagtagtccacgttgacggcggtttcagcatcgctgcaatgaacgaactcgaactgaaataattaattaaccgcgtatggtgcactctcagtacaatctgctctgatgccgcatagttaagccagccccgacacccgccaacacccgctgacgcgccctgacgggcttgtctgctcccggcatccgcttacagacaagctgtgaccgtctccgggagctcatgtgtcagaggttttcacaagttgcaggaccacttctgcgctcggcccttccggctggctggtttattgctgataaatctggagccggtgagcgtgggtctcgcggtatcattgcagcactggggccagatggtaagccctcccgtatcgtagttatctacacgacggggagtcaggcaactatggatgaacgaaatagacagatcgctgagataggtgcctcactgattaagcattggtaactgtcagaccaagtttactcatatatactttagattgatttaaaacttcatttttaatttaaaaggatctaggtgaagatcctttttgataatctcatgaccaaaatcccttaacgtgagttttcgttccactgagcgtcagaccccgtagaaaagatcaaaggatcttcttgagatcctttttttctgcgcgtaatctgctgcttgcaaacaaaaaaaccaccgctaccagcggtggtttgtttgccggatcaagagctaccaactctttttccgaaggtaactggcttcagcagagcgcagataccaaatactgtccttctagtgtagccgtagttaggccaccacttcaagaactctgtagcaccgcctacatacctcgctctgctaatcctgttaccagtggctgctgccagtggcgataagtcgtgtcttaccgggttggactcaagacgatagttaccggataaggcgcagcggtcgggctgaacggggggttcgtgcacacagcccagcttggagcgaacgacctacaccgaactgagatacctacagcgtgagctatgagaaagcgccacgcttcccgaagggagaaaggcggacaggtatccggtaagcggcagggtcggaacaggagagcgcacgagggagcttccagggggaaacgcctggtatctttatagtcctgtcgggtttcgccacctctgacttgagcgtcgatttttgtgatgctcgtcaggggggcggagcctatggaaaaacgccagcaacgcggcctttttacggttcctggccttttgctggccttttgctcacatggctcgacagatcttcaatattggccattagccatattattcattggttatatagcataaatcaatattggctattggccattgcatacgttgtatctatatcataatatgtacatttatattggctcatgtccaatatgaccgccatgttggcattgattattgactagttattaatagtaatcaattacggggtcattagttcatagcccatatatggagttccgcgttacataacttacggtaaatggcccgcctggctgaccgcccaacgacccccgcccattgacgtcaataatgacgtatgttcccatagtaacgccaatagggactttccattgacgtcaatgggtggagtatttacggtaaactgcccacttggcagtacatcaagtgtatcatatgccaagtccgccccctattgacgtcaatgacggtaaatggcccgcctggcattatgcccagtacatgaccttacgggactttcctacttggcagtacatctacgtattagtcatcgctattaccatggtgatgcggttttggcagtacaccaatgggcgtggatagcggtttgactcacggggatttccaagtctccaccccattgacgtcaatgggagtttgttttggcaccaaaatcaacgggactttccaaaatgtcgtaacaactgcgatcgcccgccccgttgacgcaaatgggcggtaggcgtgtacggtgggaggtctatataagcagagctcgtttagtgaaccgtcagatcactagaagctttattgcggtagtttatcacagttaaattgctaacgcagtcagtgcttctgacacaacagtctcgaacttaagctgcagtgactctcttaaggtagccttgcagaagttggtcgtgaggcactgggcaggtaagtatcaaggttacaagacaggtttaaggagaccaatagaaactgggcttgtcgagacagagaagactcttgcgtttctgataggcacctattggtcttactgacatccactttgcctttctctccacaggtgtccactcccagttcaattacagctcttaaggctagagtacttaatacgactcactataggctagcctcgagacgcgtggtacc

SEQ ID NO: 12 - DNA, 5160 bp, synthetic construct
  source 1..5160: mol_type = other DNA
  misc_feature 1..5160: note = pPAL-N
ggtaccatgtctgataatggaccccaaaatcagcgaaatgcaccccgcattacgtttggtggaccctcagattcaactggcagtaaccagaatggagaacgcagtggggcgcgatcaaaacaacgtcggccccaaggtttacccaataatactgcgtcttggttcaccgctctcactcaacatggcaaggaagaccttaaattccctcgaggacaaggcgttccaattaacaccaatagcagtccagatgaccaaattggctactaccgaagagctaccagacgaattcgtggtggtgacggtaaaatgaaagatctcagtccaagatggtatttctactacctaggaactgggccagaagctggacttccctatggtgctaacaaagacggcatcatatgggttgcaactgagggagccttgaatacaccaaaagatcacattggcacccgcaatcctgctaacaatgctgcaatcgtgctacaacttcctcaaggaacaacattgccaaaaggcttctacgcagaagggagcagaggcggcagtcaagcctcttctcgttcctcatcacgtagtcgcaacagttcaagaaattcaactccaggcagcagtaggggaacttctcctgctagaatggctggcaatggcggtgatgctgctcttgctttgctgctgcttgacagattgaaccagcttgagagcaaaatgtctggtaaaggccaacaacaacaaggccaaactgtcactaagaaatctgctgctgaggcttctaagaagcctcggcaaaaacgtactgccactaaagcatacaatgtaacacaagctttcggcagacgtggtccagaacaaacccaaggaaattttggggaccaggaactaatcagacaaggaactgattacaaacattggccgcaaattgcacaatttgcccccagcgcttcagcgttcttcggaatgtcgcgcattggcatggaagtcacaccttcgggaacgtggttgacctacacaggtgccatcaaattggatgacaaagatccaaatttcaaagatcaagtcattttgctgaataagcatattgacgcatacaaaacattcccaccaacagagcctaaaaaggacaaaaagaagaaggctgatgaaactcaagccttaccgcagagacagaagaaacagcaaactgtgactcttcttcctgctgcagatttggatgatttctccaaacaattgcaacaatccatgagcagtgctgactcaactcaggcctaatctagagtcgacccgggcggccgcttccctttagtgagggttaatgcttcgagcagacatgataagatacattgatgagtttggacaaaccacaactagaatgcagtgaaaaaaatgctttatttgtgaaatttgtgatgctattgctttatttgtaaccattataagctgcaataaacaagttaacaacaacaattgcattcattttatgtttcaggttcagggggagatgtgggaggttttttaaagcaagtaaaacctctacaaatgtggtaaaatccgataaggatcgatccgggctggcgtaatagcgaagaggcccgcaccgatcgcccttcccaacagttgcgcagcctgaatggcgaatggacgcgccctgtagcggcgcattaagcgcggcgggtgtggtggttacgcgcagcgtgaccgctacacttgccagcgttaattaagtgctggagaatattcggcaaggtctgaaccgtcccagccatcgccatgaaagggttaggggctgtatgagcctgtttgttgctggggtaacaatatttgcacaatacggtcccctcgcccctctggggagagggttagggtgaggggaaaagcgccccccctgccgcagcctgctccggtcggacctggcaactatagctactcacagccaggttgattataataaccgtttatctgttcgtactgtttactaaaacgacgaatcgcctgattttcaggcacaacaagcatcaacaataaggattaaagctatgggttttctttccggtaagcgcattctggtaaccggtgttgccagcaaactatccatcgcctacggtatcgctcaggcgatgcaccgcgaaggagctgaactggcattcacctaccagaacgacaaactgaaaggccgcgtagaagaatttgccgctcaattgggttctgacatcgttctgcagtgcgatgttgcagaagatgccagcatcgacaccatgttcgctgaactggggaaagtttggccgaaatttgacggtttcgtacactctattggttttgcacctggcgatcagctggatggtgactatgttaacgccgttacccgtgaaggcttcaaaattgcccacgacatcagctcctacagcttcgttgcaatggcaaaagcttgccgctccatgctgaatccgggttctgccctgctgaccctttcctaccttggcgctgagcgcgctatcccgaactacaacgttatgggtctggcaaaagcgtctctggaagcgaacgtgcgctatatggcgaacgcgatgggtccggaaggtgtgcgtgttaacgccatctctgctggtccgatccgtactctggcggcttccggtatcaaagacttccgcaaaatgctggctcattgcgaagccgttaccccgattcgccgtaccgttactattgaagatgtgggtaactctgcggcattcctgtgctccgatctctctgccggtatctccggtgaagtagtccacgttgacggcggtttcagcatcgctgcaatgaacgaactcgaactgaaataattaattaaccgcgtatggtgcactctcagtacaatctgctctgatgccgcatagttaagccagccccgacacccgccaacacccgctgacgcgccctgacgggcttgtctgctcccggcatccgcttacagacaagctgtgaccgtctccgggagctcatgtgtcagaggttttcacaagttgcaggaccacttctgcgctcggcccttccggctggctggtttattgctgataaatctggagccggtgagcgtgggtctcgcggtatcattgcagcactggggccagatggtaagccctcccgtatcgtagttatctacacgacggggagtcaggcaactatggatgaacgaaatagacagatcgctgagataggtgcctcactgattaagcattggtaactgtcagaccaagtttactcatatatactttagattgatttaaaacttcatttttaatttaaaaggatctaggtgaagatcctttttgataatctcatgaccaaaatcccttaacgtgagttttcgttccactgagcgtcagaccccgtagaaaagatcaaaggatcttcttgagatcctttttttctgcgcgtaatctgctgcttgcaaacaaaaaaaccaccgctaccagcggtggtttgtttgccggatcaagagctaccaactctttttccgaaggtaactggcttcagcagagcgcagataccaaatactgtccttctagtgtagccgtagttaggccaccacttcaagaactctgtagcaccgcctacatacctcgctctgctaatcctgttaccagtggctgctgccagtggcgataagtcgtgtcttaccgggttggactcaagacgatagttaccggataaggcgcagcggtcgggctgaacggggggttcgtgcacacagcccagcttggagcgaacgacctacaccgaactgagatacctacagcgtgagctatgagaaagcgccacgcttcccgaagggagaaaggcggacaggtatccggtaagcggcagggtcggaacaggagagcgcacgagggagcttccagggggaaacgcctggtatctttatagtcctgtcgggtttcgccacctctgacttgagcgtcgatttttgtgatgctcgtcaggggggcggagcctatggaaaaacgccagcaacgcggcctttttacggttcctggccttttgctggccttttgctcacatggctcgacagatcttcaatattggccattagccatattattcattggttatatagcataaatcaatattggctattggccattgcatacgttgtatctatatcataatatgtacatttatattggctcatgtccaatatgaccgccatgttggcattgattattgactagttattaatagtaatcaattacggggtcattagttcatagcccatatatggagttccgcgttacataacttacggtaaatggcccgcctggctgaccgcccaacgacccccgcccattgacgtcaataatgacgtatgttcccatagtaacgccaatagggactttccattgacgtcaatgggtggagtatttacggtaaactgcccacttggcagtacatcaagtgtatcatatgccaagtccgccccctattgacgtcaatgacggtaaatggcccgcctggcattatgcccagtacatgaccttacgggactttcctacttggcagtacatctacgtattagtcatcgctattaccatggtgatgcggttttggcagtacaccaatgggcgtggatagcggtttgactcacggggatttccaagtctccaccccattgacgtcaatgggagtttgttttggcaccaaaatcaacgggactttccaaaatgtcgtaacaactgcgatcgcccgccccgttgacgcaaatgggcggtaggcgtgtacggtgggaggtctatataagcagagctcgtttagtgaaccgtcagatcactagaagctttattgcggtagtttatcacagttaaattgctaacgcagtcagtgcttctgacacaacagtctcgaacttaagctgcagtgactctcttaaggtagccttgcagaagttggtcgtgaggcactgggcaggtaagtatcaaggttacaagacaggtttaaggagaccaatagaaactgggcttgtcgagacagagaagactcttgcgtttctgataggcacctattggtcttactgacatccactttgcctttctctccacaggtgtccactcccagttcaattacagctcttaaggctagagtacttaatacgactcactataggctagcctcgagacgcgtggtacc

SEQ ID NO: 13 - DNA, 5160 bp, synthetic construct
  source 1..5160: mol_type = other DNA
  misc_feature 1..5160: note = pPAL-N (codon-optimized N gene)
ggtaccatgtccgataacggcccccagaaccaacgcaatgcccctcggattacattcggcggacccagcgactccaccgggagcaaccaaaacggcgagcgcagcggagcacggtctaagcagagaaggcctcaggggctgccaaataacactgcttcttggttcactgctctgacacagcatggaaaagaggacctcaaatttccccggggccagggcgttcccatcaacactaactcttccccagatgaccagatcgggtattaccgcagggctactcggagaatcaggggcggggacgggaaaatgaaggatctcagcccaaggtggtacttttattatctcggcacagggcctgaagccggactgccctatggagctaacaaagacggcattatttgggtggcaactgagggcgccctgaacaccccaaaagatcatatcggaacccgcaatcctgccaataacgctgccattgtgctccagctgcctcaggggacaacactgcccaaagggttctacgcagaaggcagccgcgggggatctcaggcaagctctcggtcctcttctagatccagaaacagctctaggaattccaccccagggtcctccagaggaacatccccagctagaatggcaggaaatggaggcgacgctgcactggcactgctgctgctggacagactgaaccagctcgagagcaaaatgtctggaaaggggcagcagcagcaagggcagaccgtcaccaagaagagcgccgccgaagctagcaagaaacctaggcagaaaaggaccgcaacaaaggcctataatgtgacccaagccttcggacgccgcggcccagaacagacccaaggcaatttcggcgaccaggagctgatccggcaaggcactgattacaagcactggccacagattgctcaattcgcccccagcgctagcgccttctttggaatgtcccggattggcatggaggtgacaccatctggcacttggctcacctacacaggggctatcaagctcgatgacaaagatcccaattttaaagaccaggtcatcctgctgaataaacacatcgatgcatacaagacttttcctcctactgaacccaaaaaggataagaagaagaaagcagatgagacccaggccctgccccagagacaaaagaagcagcagaccgttacactgctccctgccgccgacctcgacgatttttccaagcagctgcagcaatctatgagcagcgccgactccacccaggcctagtctagagtcgacccgggcggccgcttccctttagtgagggttaatgcttcgagcagacatgataagatacattgatgagtttggacaaaccacaactagaatgcagtgaaaaaaatgctttatttgtgaaatttgtgatgctattgctttatttgtaaccattataagctgcaataaacaagttaacaacaacaattgcattcattttatgtttcaggttcagggggagatgtgggaggttttttaaagcaagtaaaacctctacaaatgtggtaaaatccgataaggatcgatccgggctggcgtaatagcgaagaggcccgcaccgatcgcccttcccaacagttgcgcagcctgaatggcgaatggacgcgccctgtagcggcgcattaagcgcggcgggtgtggtggttacgcgcagcgtgaccgctacacttgccagcgttaattaagtgctggagaatattcggcaaggtctgaaccgtcccagccatcgccatgaaagggttaggggctgtatgagcctgtttgttgctggggtaacaatatttgcacaatacggtcccctcgcccctctggggagagggttagggtgaggggaaaagcgccccccctgccgcagcctgctccggtcggacctggcaactatagctactcacagccaggttgattataataaccgtttatctgttcgtactgtttactaaaacgacgaatcgcctgattttcaggcacaacaagcatcaacaataaggattaaagctatgggttttctttccggtaagcgcattctggtaaccggtgttgccagcaaactatccatcgcctacggtatcgctcaggcgatgcaccgcgaaggagctgaactggcattcacctaccagaacgacaaactgaaaggccgcgtagaagaatttgccgctcaattgggttctgacatcgttctgcagtgcgatgttgcagaagatgccagcatcgacaccatgttcgctgaactggggaaagtttggccgaaatttgacggtttcgtacactctattggttttgcacctggcgatcagctggatggtgactatgttaacgccgttacccgtgaaggcttcaaaattgcccacgacatcagctcctacagcttcgttgcaatggcaaaagcttgccgctccatgctgaatccgggttctgccctgctgaccctttcctaccttggcgctgagcgcgctatcccgaactacaacgttatgggtctggcaaaagcgtctctggaagcgaacgtgcgctatatggcgaacgcgatgggtccggaaggtgtgcgtgttaacgccatctctgctggtccgatccgtactctggcggcttccggtatcaaagacttccgcaaaatgctggctcattgcgaagccgttaccccgattcgccgtaccgttactattgaagatgtgggtaactctgcggcattcctgtgctccgatctctctgccggtatctccggtgaagtagtccacgttgacggcggtttcagcatcgctgcaatgaacgaactcgaactgaaataattaattaaccgcgtatggtgcactctcagtacaatctgctctgatgccgcatagttaagccagccccgacacccgccaacacccgctgacgcgccctgacgggcttgtctgctcccggcatccgcttacagacaagctgtgaccgtctccgggagctcatgtgtcagaggttttcacaagttgcaggaccacttctgcgctcggcccttccggctggctggtttattgctgataaatctggagccggtgagcgtgggtctcgcggtatcattgcagcactggggccagatggtaagccctcccgtatcgtagttatctacacgacggggagtcaggcaactatggatgaacgaaatagacagatcgctgagataggtgcctcactgattaagcattggtaactgtcagaccaagtttactcatatatactttagattgatttaaaacttcatttttaatttaaaaggatctaggtgaagatcctttttgataatctcatgaccaaaatcccttaacgtgagttttcgttccactgagcgtcagaccccgtagaaaagatcaaaggatcttcttgagatcctttttttctgcgcgtaatctgctgcttgcaaacaaaaaaaccaccgctaccagcggtggtttgtttgccggatcaagagctaccaactctttttccgaaggtaactggcttcagcagagcgcagataccaaatactgtccttctagtgtagccgtagttaggccaccacttcaagaactctgtagcaccgcctacatacctcgctctgctaatcctgttaccagtggctgctgccagtggcgataagtcgtgtcttaccgggttggactcaagacgatagttaccggataaggcgcagcggtcgggctgaacggggggttcgtgcacacagcccagcttggagcgaacgacctacaccgaactgagatacctacagcgtgagctatgagaaagcgccacgcttcccgaagggagaaaggcggacaggtatccggtaagcggcagggtcggaacaggagagcgcacgagggagcttccagggggaaacgcctggtatctttatagtcctgtcgggtttcgccacctctgacttgagcgtcgatttttgtgatgctcgtcaggggggcggagcctatggaaaaacgccagcaacgcggcctttttacggttcctggccttttgctggccttttgctcacatggctcgacagatcttcaatattggccattagccatattattcattggttatatagcataaatcaatattggctattggccattgcatacgttgtatctatatcataatatgtacatttatattggctcatgtccaatatgaccgccatgttggcattgattattgactagttattaatagtaatcaattacggggtcattagttcatagcccatatatggagttccgcgttacataacttacggtaaatggcccgcctggctgaccgcccaacgacccccgcccattgacgtcaataatgacgtatgttcccatagtaacgccaatagggactttccattgacgtcaatgggtggagtatttacggtaaactgcccacttggcagtacatcaagtgtatcatatgccaagtccgccccctattgacgtcaatgacggtaaatggcccgcctggcattatgcccagtacatgaccttacgggactttcctacttggcagtacatctacgtattagtcatcgctattaccatggtgatgcggttttggcagtacaccaatgggcgtggatagcggtttgactcacggggatttccaagtctccaccccattgacgtcaatgggagtttgttttggcaccaaaatcaacgggactttccaaaatgtcgtaacaactgcgatcgcccgccccgttgacgcaaatgggcggtaggcgtgtacggtgggaggtctatataagcagagctcgtttagtgaaccgtcagatcactagaagctttattgcggtagtttatcacagttaaattgctaacgcagtcagtgcttctgacacaacagtctcgaacttaagctgcagtgactctcttaaggtagccttgcagaagttggtcgtgaggcactgggcaggtaagtatcaaggttacaagacaggtttaaggagaccaatagaaactgggcttgtcgagacagagaagactcttgcgtttctgataggcacctattggtcttactgacatccactttgcctttctctccacaggtgtccactcccagttcaattacagctcttaaggctagagtacttaatacgactcactataggctagcctcgagacgcgtggtacc

SEQ ID NO: 14 - DNA, 12 bp, synthetic construct
  source 1..12: mol_type = other DNA
  misc_feature 1..12: note = sequence encoding furin cleavage site at protein S
cctcggcgggca

SEQ ID NO: 15 - DNA, 12 bp, synthetic construct
  source 1..12: mol_type = other DNA
  misc_feature 1..12: note = sequence encoding modified furin cleavage site
ccaggcggcagc

SEQ ID NO: 16 - DNA, 312 bp, synthetic construct
  source 1..312: mol_type = other DNA
  misc_feature 1..312: note = promoter of the FabI gene
gtgctggagaatattcggcaaggtctgaaccgtcccagccatcgccatgaaagggttaggggctgtatgagcctgtttgttgctggggtaacaatatttgcacaatacggtcccctcgcccctctggggagagggttagggtgaggggaaaagcgccccccctgccgcagcctgctccggtcggacctggcaactatagctactcacagccaggttgattataataaccgtttatctgttcgtactgtttactaaaacgacgaatcgcctgattttcaggcacaacaagcatcaacaataaggattaaagct

SEQ ID NO: 17 - protein, 262 aa, synthetic construct
  REGION 1..262: note = enoyl-acyl carrier protein (ACP) reductase
MGFLSGKRILVTGVASKLSIAYGIAQAMHREGAELAFTYQNDKLKGRVEEFAAQLGSDIVLQCDVAEDASIDTMFAELGKVWPKFDGFVHSIGFAPGDQLDGDYVNAVTREGFKIAHDISSYSFVAMAKACRSMLNPGSALLTLSYLGAERAIPNYNVMGLAKASLEANVRYMANAMGPEGVRVNAISAGPIRTLAASGIKDFRKMLAHCEAVTPIRRTVTIEDVGNSAAFLCSDLSAGISGEVVHVDGGFSIAAMNELELK

SEQ ID NO: 18 - DNA, 20 bp, synthetic construct
  source 1..20: mol_type = other DNA
  misc_feature 1..20: note = N1-F forward primer
gaccccaaaatcagcgaaat

SEQ ID NO: 19 - DNA, 24 bp, synthetic construct
  source 1..24: mol_type = other DNA
  misc_feature 1..24: note = N1-R reverse primer
tctggttactgccagttgaatctg

SEQ ID NO: 20 - DNA, 24 bp, synthetic construct
  source 1..24: mol_type = other DNA
  modified_base 1: mod_base = OTHER; note = 6-Carboxyfluorescein (6-FAM)
  modified_base 24: mod_base = OTHER; note = Black Hole Quencher-1 (BHQ-1)
accccgcattacgtttggtggacc

SEQ ID NO: 21 - DNA, 25 bp, synthetic construct
  source 1..25: mol_type = other DNA
  misc_feature 1..25: note = forward primer ACT_F_1005-1029
cagcacaatgaagatcaagatcatc

SEQ ID NO: 22 - DNA, 22 bp, synthetic construct
  source 1..22: mol_type = other DNA
  misc_feature 1..22: note = Reverse primer ACT_R_1135-1114
cggactcatcgtactcctgctt

SEQ ID NO: 23 - DNA, 25 bp, synthetic construct
  source 1..25: mol_type = other DNA
  modified_base 1: mod_base = OTHER; note = 5'-Dichloro-dimethoxy-fluorescein (JOE)
  modified_base 25: mod_base = OTHER; note = Black Hole Quencher-1 (BHQ-1)
tcgctgtccaccttccagcagatgt

SEQ ID NO: 24 - protein, 1268 aa, synthetic construct
  REGION 1..1268: note = S protein Omicron Subvariant BA.4 (GenBank: UUB32912.1)
MFGFLVLLPLVSSQCVNLITRTQSYTNSFTRGVYYPDKVFRSSVLHSTQDLFLPFFSNVTWFHAISGTNGTKRFDNPVLPFNDGVYFASTEKSNIIRGWIFGTTLDSKTQSLLIVNNATNVVIKVCEFQFCNDPFLDVYYHKNNKSWMESEFRVYSSANNCTFEYVSQPFLMDLEGKQGNFKNLREFVFKNIDGYFKIYSKHTPINLGRDLPQGFSALEPLVDLPIGINITRFQTLLALHRSYLTPGDSSSGWTAGAAAYYVGYLQPRTFLLKYNENGTITDAVDCALDPLSETKCTLKSFTVEKGIYQTSNFRVQPTESIVRFPNITNLCPFDEVFNATRFASVYAWNRKRISNCVADYSVLYNFAPFFAFKCYGVSPTKLNDLCFTNVYADSFVIRGNEVSQIAPGQTGNIADYNYKLPDDFTGCVIAWNSNKLDSKVGGNYNYRYRLFRKSNLKPFERDISTEIYQAGNKPCNGVAGVNCYFPLQSYGFRPTYGVGHQPYRVVVLSFELLHAPATVCGPKKSTNLVKNKCVNFNFNGLTGTGVLTESNKKFLPFQQFGRDIADTTDAVRDPQTLEILDITPCSFGGVSVITPGTNTSNQVAVLYQGVNCTEVPVAIHADQLTPTWRVYSTGSNVFQTRAGCLIGAEYVNNSYECDIPIGAGICASYQTQTKSHRRARSVASQSIIAYTMSLGAENSVAYSNNSIAIPTNFTISVTTEILPVSMTKTSVDCTMYICGDSTECSNLLLQYGSFCTQLKRALTGIAVEQDKNTQEVFAQVKQIYKTPPIKYFGGFNFSQILPDPSKPSKRSFIEDLLFNKVTLADAGFIKQYGDCLGDIAARDLICAQKFNGLTVLPPLLTDEMIAQYTSALLAGTITSGWTFGAGAALQIPFAMQMAYRFNGIGVTQNVLYENQKLIANQFNSAIGKIQDSLSSTASALGKLQDVVNHNAQALNTLVKQLSSKFGAISSVLNDILSRLDKVEAEVQIDRLITGRLQSLQTYVTQQLIRAAEIRASANLAATKMSECVLGQSKRVDFCGKGYHLMSFPQSAPHGVVFLHVTYVPAQEKNFTTAPAICHDGKAHFPREGVFVSNGTHWFVTQRNFYEPQIITTDNTFVSGNCDVVIGIVNNTVYDPLQPELDSFKEELDKYFKNHTSPDVDLGDISGINASVVNIQKEIDRLNEVAKNLNESLIDLQELGKYEQYIKWPWYIWLGFIAGLIAIVMVTIMLCCMTSCCSCLKGCCSCGSCCKFDEDDSEPVLKGVKLHYT

SEQ ID NO: 25 - protein, 1268 aa, synthetic construct
  REGION 1..1268: note = S protein Omicron Subvariant BA.5 (GenBank: UUB32864.1)
MFVFLVLLPLVSSQCVNLITRTQSYTNSFTRGVYYPDKVFRSSVLHSTQDLFLPFFSNVTWFHAISGTNGTKRFDNPVLPFNDGVYFASTEKSNIIRGWIFGTTLDSKTQSLLIVNNATNVVIKVCEFQFCNDPFLDVYYHKNNKSWMESEFRVYSSANNCTFEYVSQPFLMDLEGKQGNFKNLREFVFKNIDGYFKIYSKHTPINLGRDLPQGFSALEPLVDLPIGINITRFQTLLALHRSYLTPGDSSSGWTAGAAAYYVGYLQPRTFLLKYNENGTITDAVDCALDPLSETKCTLKSFTVEKGIYQTSNFRVQPTESIVRFPNITNLCPFDEVFNATRFASVYAWNRKRISNCVADYSVLYNFAPFFAFKCYGVSPTKLNDLCFTNVYADSFVIRGNEVSQIAPGQTGNIADYNYKLPDDFTGCVIAWNSNKLDSKVGGNYNYRYRLFRKSNLKPFERDISTEIYQAGNKPCNGVAGVNCYFPLQSYGFRPTYGVGHQPYRVVVLSFELLHAPATVCGPKKSTNLVKNKCVNFNFNGLTGTGVLTESNKKFLPFQQFGRDIADTTDAVRDPQTLEILDITPCSFGGVSVITPGTNTSNQVAVLYQGVNCTEVPVAIHADQLTPTWRVYSTGSNVFQTRAGCLIGAEYVNNSYECDIPIGAGICASYQTQTKSHRRARSVASQSIIAYTMSLGAENSVAYSNNSIAIPTNFTISVTTEILPVSMTKTSVDCTMYICGDSTECSNLLLQYGSFCTQLKRALTGIAVEQDKNTQEVFAQVKQIYKTPPIKYFGGFNFSQILPDPSKPSKRSFIEDLLFNKVTLADAGFIKQYGDCLGDIAARDLICAQKFNGLTVLPPLLTDEMIAQYTSALLAGTITSGWTFGAGAALQIPFAMQMAYRFNGIGVTQNVLYENQKLIANQFNSAIGKIQDSLSSTASALGKLQDVVNHNAQALNTLVKQLSSKFGAISSVLNDILSRLDKVEAEVQIDRLITGRLQSLQTYVTQQLIRAAEIRASANLAATKMSECVLGQSKRVDFCGKGYHLMSFPQSAPHGVVFLHVTYVPAQEKNFTTAPAICHDGKAHFPREGVFVSNGTHWFVTQRNFYEPQIITTDNTFVSGNCDVVIGIVNNTVYDPLQPELDSFKEELDKYFKNHTSPDVDLGDISGINASVVNIQKEIDRLNEVAKNLNESLIDLQELGKYEQYIKWPWYIWLGFIAGLIAIVMVTIMLCCMTSCCSCLKGCCSCGSCCKFDEDDSEPVLKGVKLHYT

SEQ ID NO: 26 - protein, 1270 aa, synthetic construct
  REGION 1..1270: note = S protein Omicron Subvariant BA2.12.1 (GenBank: UUB32948.1)
MFVFLVLLPLVSSQCVNLITRTQSYTNSFTRGVYYPDKVFRSSVLHSTQDLFLPFFSNVTWFHAIHVSGTNGTKRFDNPVLPFNDGVYFASTEKSNIIRGWIFGTTLDSKTQSLLIVNNATNVVIKVCEFQFCNDPFLDVYYHKNNKSWMESEFRVYSSANNCTFEYVSQPFLMDLEGKQGNFKNLREFVFKNIDGYFKIYSKHTPINLGRDLPQGFSALEPLVDLPIGINITRFQTLLALHRSYLTPGDSSSGWTAGAAAYYVGYLQPRTFLLKYNENGTITDAVDCALDPLSETKCTLKSFTVEKGIYQTSNFRVQPTESIVRFPNITNLCPFDEVFNATRFASVYAWNRKRISNCVADYSVLYNFAPFFAFKCYGVSPTKLNDLCFTNVYADSFVIRGNEVSQIAPGQTGNIADYNYKLPDDFTGCVIAWNSNKLDSKVGGNYNYQYRLFRKSNLKPFERDISTEIYQAGNKPCNGVAGFNCYFPLRSYGFRPTYGVGHQPYRVVVLSFELLHAPATVCGPKKSTNLVKNKCVNFNFNGLTGTGVLTESNKKFLPFQQFGRDIADTTDAVRDPQTLEILDITPCSFGGVSVITPGTNTSNQVAVLYQGVNCTEVPVAIHADQLTPTWRVYSTGSNVFQTRAGCLIGAEYVNNSYECDIPIGAGICASYQTQTKSHRRARSVASQSIIAYTMSLGAENLVAYSNNSIAIPTNFTISVTTEILPVSMTKTSVDCTMYICGDSTECSNLLLQYGSFCTQLKRALTGIAVEQDKNTQEVFAQVKQIYKTPPIKYFGGFNFSQILPDPSKPSKRSFIEDLLFNKVTLADAGFIKQYGDCLGDIAARDLICAQKFNGLTVLPPLLTDEMIAQYTSALLAGTITSGWTFGAGAALQIPFAMQMAYRFNGIGVTQNVLYENQKLIANQFNSAIGKIQDSLSSTASALGKLQDVVNHNAQALNTLVKQLSSKFGAISSVLNDILSRLDKVEAEVQIDRLITGRLQSLQTYVTQQLIRAAEIRASANLAATKMSECVLGQSKRVDFCGKGYHLMSFPQSAPHGVVFLHVTYVPAQEKNFTTAPAICHDGKAHFPREGVFVSNGTHWFVTQRNFYEPQIITTDNTFVSGNCDVVIGIVNNTVYDPLQPELDSFKEELDKYFKNHTSPDVDLGDISGINASVVNIQKEIDRLNEVAKNLNESLIDLQELGKYEQYIKWPWYIWLGFIAGLIAIVMVTIMLCCMTSCCSCLKGCCSCGSCCKFDEDDSEPVLKGVKLHYT

SEQ ID NO: 27 - protein, 1270 aa, synthetic construct
  REGION 1..1270: note = S protein Omicron Subvariant BA2.9.1 (GenBank: UUA48363.1)
MFVFLVLLPLVSSQCVNLITRTQSYTNSFTRGVYYPDKVFRSSVLHSTQDLFLPFFSNVTWFHAIHVSGTNGTKRFDNPVLPFNDGVYFASTEKSNIIRGWIFGTTLDSKTQSLLIVNNATNVVIKVCEFQFCNDPFLDVYYHKNNKSWMESEFRVYSSANNCTFEYVSQPFLMDLEGKQGNFKNLREFVFKNIDGYFKIYSKHTPINLGRDLPQGFSALEPLVDLPIGINITRFQTLLALHRSYLTPGDSSSGWTAGAAAYYVGYLQPRTFLLKYNENGTITDAVDCALDPLSETKCTLKSFTVEKGIYQTSNFRVQPTESIVRFPNITNLCPFDEVFNATRFASVYAWNRKRISNCVADYSVLYNFAPFFAFKCYGVSPTKLNDLCFTNVYADSFVIRGNEVSQIAPGQTGNIADYNYKLPDDFTGCVIAWNSNKLDSKVGGNYNYLYRLFRKSNLKPFERDISTEIYQAGNKPCNGVAGFNCYFPLRSYGFRPTYGVGHQPYRVVVLSFELLHAPATVCGPKKSTNLVKNKCVNFNFNGLTGTGVLTESNKKFLPFQQFGRDIADTTDAVRDPQTLEILDITPCSFGGVSVITPGTNTSNQVAVLYQGVNCTEVPVAIHADQLTPTWRVYSTGSNVFQTRAGCLIGAEYVNNSYECDIPIGAGICASYQTQTKSHRRARSVASQSIIAYTMSLGAENSVAYSNNSIAIPTNFTISVTTEILPVSMTKTSVDCTMYICGDSTECSNLLLQYGSFCTQLKRALTGIAVEQDKNTQEVFAQVKQIYKTPPIKYFGGFNFSQILPDPSKPSKRSFIEDLLFNKVTLADAGFIKQYGDCLGDIAARDLICAQKFNGLTVLPPLLTDEMIAQYTSALLAGTITSGWTFGAGAALQIPFAMQMAYRFNGIGVTQNVLYENQKLIANQFNSAIGKIQDSLSSTASALGKLQDVVNHNAQALNTLVKQLSSKFGAISSVLNDILSRLDKVEAEVQIDRLITGRLQSLQTYVTQQLIRAAEIRASANLAATKMSECVLGQSKRVDFCGKGYHLMSFPQSAPHGVVFLHVTYVPAQEKNFTTAPAICHDGKAHFPREGVFVSNGTHWFVTQRNFYEPQIITTDNTFVSGNCDVVIGIVNNTVYDPLQPELDSFKEELDKYFKNHTSPDVDLGDISGINASVVNIQKEIDRLNEVAKNLNESLIDLQELGKYEQYIKWPWYIWLGFIAGLIAIVMVTIMLCCMTSCCSCLKGCCSCGSCCKFDEDDSEPVLKGVKLHYT

SEQ ID NO: 28 - protein, 194 aa, synthetic construct
  REGION 1..194: note = receptor-binding domain (RBD)
NITNLCPFGEVFNATRFASVYAWNRKRISNCVADYSVLYNSASFSTFKCYGVSPTKLNDLCFTNVYADSFVIRGDEVRQIAPGQTGKIADYNYKLPDDFTGCVIAWNSNNLDSKVGGNYNYLYRLFRKSNLKPFERDISTEIYQAGSTPCNGVEGFNCYFPLQSYGFQPTNGVGYQPYRVVVLSFELLHAPATV

SEQ ID NO: 29 - protein, 416 aa, synthetic construct
  REGION 1..416: note = N protein Omicron Subvariant BA.4 (GenBank: UUB32920.1)
MSDNGPQNQRNALRITFGGPSDSTGSNQNGGARSKQRRPQGLPNNTASWFTALTQHGKEDLKFPRGQGVPINTNSSPDDQIGYYRRATRRIRGGDGKMKDLSPRWYFYYLGTGPEAGLPYGANKDGIIWVATEGALNTPKDHIGTRNSANNAAIVLQLPQGTTLPKGFYAEGSRGGSQASSRSSSRSRNSSRNSTPGSSKRTSPARMAGNGGDAALALLLLDRLNQLESKMSGKGQQQQGQTVTKKSAAEASKKPRQKRTATKAYNVTQAFGRRGPEQTQGNFGDQELIRQGTDYKHWPQIAQFAPSASAFFGMSRIGMEVTPSGTWLTYTGAIKLDDKDPNFKDQVILLNKHIDAYKTFPPTEPKKDKKKKADETQALPQRQKKQQTVTLLPAADLDDFSKQLQQSMSRADSTQA

SEQ ID NO: 30 - protein, 416 aa, synthetic construct
  REGION 1..416: note = N protein Omicron Subvariant BA.5 (GenBank: UUB32872.1)
MSDNGPQNQRNALRITFGGPSDSTGSNQNGGARSKQRRPQGLPNNTASWFTALTQHGKEDLKFPRGQGVPINTNSSPDDQIGYYRRATRRIRGGDGKMKDLSPRWYFYYLGTGPEAGLPYGANKDGIIWVATEGALNTPKDHIGTRNPANNAAIVLQLPQGTTLPKGFYAEGSRGGSQASSRSSSRSRNSSRNSTPGSSKRTSPARMAGNGGDAALALLLLDRLNQLESKMSGKGQQQQGQTVTKKSAAEASKKPRQKRTATKAYNVTQAFGRRGPEQTQGNFGDQELIRQGTDYKHWPQIAQFAPSASAFFGMSRIGMEVTPSGTWLTYTGAIKLDDKDPNFKDQVILLNKHIDAYKTFPPTEPKKDKKKKADETQALPQRQKKQQTVTLLPAADLDDFSKQLQQSMSRADSTQA

SEQ ID NO: 31 - protein, 416 aa, synthetic construct; identical to SEQ ID NO: 30
  REGION 1..416: note = N protein Omicron Subvariant BA2.12.1 (GenBank: UUB32956.1)

SEQ ID NO: 32 - protein, 416 aa, synthetic construct; identical to SEQ ID NO: 30
  REGION 1..416: note = N protein Omicron Subvariant BA2.9.1 (GenBank: UUA48371.1)